European Patent Application EP 4 166 656 A1, published April 19, 2023. Title: Recombinant Herpes Simplex Virus Containing Expression Cassette Expressing a Fused Protein of Tumor Cell-targeting Domain and Extracellular Damain of HVEM and Use of the Same. Applicant: KOREA, Gencellmed. The sequence listing filed with the application follows.

SEQUENCE LISTING (46 sequences)

SEQ ID NO: 1 - protein, 904 aa, Artificial Sequence
  gB
MHQGAPSWGRRWFVVWALLGLTLGVLVASAAPSSPGTPGVAAATQAANGGPATPAPPALGAAPTGDPKPKKNKKPKNPTPPRPAGDNATVAAGHATLREHLRDIKAENTDANFYVCPPPTGATVVQFEQPRRCPTRPEGQNYTEGIAVVFKENIAPYKFKATMYYKDVTVSQVWFGHRYSQFMGIFEDRAPVPFEEVIDKINAKGVCRSTAKYVRNNLETTAFHRDDHETDMELKPANAATRTSRGWHTTDLKYNPSRVEAFHRYGTTVNCIVEEVDARSVYPYDEFVLATGDFVYMSPFYGYREGSHTEHTSYTADRFKQVDGFYARDLTTKARATAPTTRNLLTTPKFTVAWDWVPKRPSVCTMTKWQEVDEMLRSEYGGSFRFSSDAISTTFTTNLTEYPLSRVDLGDCIGKDARDAMDRIFARRYNATHIKVGQPQYYLANGGFLIAYQPLLSNTLAELYVREHLREQSRKPPNPTPPPPGASANASVERIKTTSSIEFARLQFTYNHIQRHVNDMLGRVAIAWCELQNHELTLWNEARKLNPNAIASVTVGRRVSARMLGDVMAVSTCVPVAADNVIVQNSMRISSRPGACYSRPLVSFRYEDQGPLVEGQLGENNELRLTRDAIEPCTVGHRRYFTFGGGYVYFEEYAYSHQLSRADITTVSTFIDLNITMLEDHEFVPLEVYTRHEIKDSGLLDYTEVQRRNQLHDLRFADIDTVIHADANAAMFAGLGAFFEGMGDLGRAVGKVVMGIVGGVVSAVSGVSSFMSNPFGALAVGLLVLAGLAAAFFAFRYVMRLQSNPMKALYPLTTKELKNPTNPDASGEGEEGGDFDEAKLAEAREMIRYMALVSAMERTEHKAKKKGTSALLSAKVTDMVMRKRRNTNYTQVPNKDGDADEDDL

SEQ ID NO: 2 - protein, 511 aa, Artificial Sequence
  gC
MAPGRVGLAVVLWSLLWLGAGVAGGSETASTGPTITAGAVTNASEAPTSGSPGSAASPEVTPTSTPNPNNVTQNKTTPTEPASPPTTPKPTSTPKSPPTSTPDPKPKNNTTPAKSGRPTKPPGPVWCDRRDPLARYGSRVQIRCRFRNSTRMEFRLQIWRYSMGPSPPIAPAPDLEEVLTNITAPPGGLLVYDSAPNLTDPHVLWAEGAGPGADPPLYSVTGPLPTQRLIIGEVTPATQGMYYLAWGRMDSPHEYGTWVRVRMFRPPSLTLQPHAVMEGQPFKATCTAAAYYPRNPVEFVWFEDDRQVFNPGQIDTQTHEHPDGFTTVSTVTSEAVGGQVPPRTFTCQMTWHRDSVMFSRRNATGLALVLPRPTITMEFGVRHVVCTAGCVPEGVTFAWFLGDDPSPAAKSAVTAQESCDHPGLATVRSTLPISYDYSEYICRLTGYPAGIPVLEHHGSHQPPPRDPTERQVIEAIEWVGIGIGVLAAGVLVVTAIVYVVRTSQSRQRHRR

SEQ ID NO: 3 - protein, 838 aa, Artificial Sequence
  gH
MGNGLWFVGVILLGVAWGQVHDWTEQTDPWFLDGLGMDRMYWRDTNTGRLWLPNTPDPQKPPRGFLAPPDELNLTTASLPLLRWYEERFCFVLVTTAEFPRDPGQLLYISKTYLLGRPPNASLPAPITVEPTAQPPPAVAPLKGLLHNPTASVLLRSRAWVTFSAVPDPEALTFPRGDNVATASHPSGPRDTPPPRPPVGARRHPTTELDITHLHNASTTWLATRGLLRSPGRYVYFSPSASTWPVGIWTTGELVLGCDAALVRARYGREFMGLVISMHDSPPVEVMVVPAGQTLDRVGDPADENPPGALPGPPGGPRYRVFVLGSLTRADNGSALDALRRVGGYPEEGTNYAQFLSRAYAEFFSGDAGAEQGPRPPLFWRLTGLLATSGFAFVNAAHANGAVCLSDLLGFLAHSRALAGLAARGAAGCAADSVFFNVSVLDPTARLQLEARLQHLVAEILEREQSLALHALGYQLAFVLDSPSAYDAVAPSAAHLIDALYAEFLGGRVLTTPVVHRALFYASAVLRQPFLAGVPSAVQRERARRSLLIASALCTSDVAAATNADLRTALARADHQKTLFWLPDHFSPCAASLRFDLDESVFILDALAQATRSETPVEVLAQQTHGLASTLTRWAHYNALIRAFVPEASHRCGGQSANVEPRILVPITHNASYVVTHSPLPRGIGYKLTGVDVRRPLFLTYLTATCEGSTRDIESKRLVRTQNQRDLGLVGAVFMRYTPAGEVMSVLLVDTDNTQQQIAAGPTEGAPSVFSSDVPSTALLLFPNGTVIHLLAFDTQPVAAIAPGFLAASALGVVMITAALAGILKVLRTSVPFFWRRE

SEQ ID NO: 4 - protein, 120 aa, Artificial Sequence [sequence omitted]

SEQ ID NO: 5 - protein, 107 aa, Artificial Sequence [sequence omitted]

SEQ ID NO: 6 - protein, 113 aa, Artificial Sequence
  EpCAM VL
DIQMTQSPSSLSASVGDRVTITCRSTKSLLHSNGITYLYWYQQKPGKAPKLLIYQMSNLASGVPSRFSSSGSGTDFTLTISSLQPEDFATYYCAQNLEIPRTFGQGTKVELKR

SEQ ID NO: 7 - protein, 114 aa, Artificial Sequence
  EpCAM VH
QLVQSGPGLVQPGGSVRISCAASGYTFTNYGMNWVKQAPGKGLEWMGWINTYTGESTYADSFKGRFTFSLDTSASAAYLQINSLRAEDTAVYYCARFAIKGDYWGQGTLLTVSS

SEQ ID NO: 8 - protein, 82 aa, Artificial Sequence
  HveA 82
LPSCKEDEYPVGSECCPKCSPGYRVKEACGELTGTVCEPCPPGTYIAHLNGLSKCLQCQMCDPAMGLRASRNCSRTENAVCG

SEQ ID NO: 9 - protein, 120 aa, Artificial Sequence
  leader sequence _ HveA82
MEPPGDWGPPPWRSTPRTDVLRLVLYLTFLGAPCYAPALPSCKEDEYPVGSECCPKCSPGYRVKEACGELTGTVCEPCPPGTYIAHLNGLSKCLQCQMCDPAMGLRASRNCSRTENAVCG

SEQ ID NO: 10 - protein, 87 aa, Artificial Sequence
  HveA 87
LPSCKEDEYPVGSECCPKCSPGYRVKEACGELTGTVCEPCPPGTYIAHLNGLSKCLQCQMCDPAMGLRASRNCSRTENAVCGCSPGH

SEQ ID NO: 11 - protein, 125 aa, Artificial Sequence
  leader sequence - HveA 87
MEPPGDWGPPPWRSTPRTDVLRLVLYLTFLGAPCYAPALPSCKEDEYPVGSECCPKCSPGYRVKEACGELTGTVCEPCPPGTYIAHLNGLSKCLQCQMCDPAMGLRASRNCSRTENAVCGCSPGH

SEQ ID NO: 12 - protein, 102 aa, Artificial Sequence
  HveA 102
LPSCKEDEYPVGSECCPKCSPGYRVKEACGELTGTVCEPCPPGTYIAHLNGLSKCLQCQMCDPAMGLRASRNCSRTENAVCGCSPGHFCIVQDGDHCAACRA

SEQ ID NO: 13 - protein, 140 aa, Artificial Sequence
  leader sequence - HveA 102
MEPPGDWGPPPWRSTPRTDVLRLVLYLTFLGAPCYAPALPSCKEDEYPVGSECCPKCSPGYRVKEACGELTGTVCEPCPPGTYIAHLNGLSKCLQCQMCDPAMGLRASRNCSRTENAVCGCSPGHFCIVQDGDHCAACRA

SEQ ID NO: 14 - protein, 107 aa, Artificial Sequence
  HveA 107
LPSCKEDEYPVGSECCPKCSPGYRVKEACGELTGTVCEPCPPGTYIAHLNGLSKCLQCQMCDPAMGLRASRNCSRTENAVCGCSPGHFCIVQDGDHCAACRAYATSS

SEQ ID NO: 15 - protein, 145 aa, Artificial Sequence
  leader sequence - HveA 107
MEPPGDWGPPPWRSTPRTDVLRLVLYLTFLGAPCYAPALPSCKEDEYPVGSECCPKCSPGYRVKEACGELTGTVCEPCPPGTYIAHLNGLSKCLQCQMCDPAMGLRASRNCSRTENAVCGCSPGHFCIVQDGDHCAACRAYATSS

SEQ ID NO: 16 - protein, 369 aa, Artificial Sequence
  gD (ASM47818)
KYALADASLKMADPNRFRGKDLPVLDQLTDPPGVRRVYHIQAGLPDPFQPPSLPITVYYAVLERACRSVLLNAPSEAPQIVRGASEDVRKQPYNLTIAWFRMGGNCAIPITVMEYTECSYNKSLGACPIRTQPRWNYYDSFSAVSEDNLGFLMHAPAFETAGTYLRLVKINDWTEITQFILEHRAKGSCKYALPLRIPPSACLSPQAYQQGVTVDSIGMLPRFIPENQRTVAVYSLKIAGWHGPKAPYTSTLLPPELSETPNATQPELAPEDPEDSALLEDPVGTVAPQIPPNWHIPSIQDAATPYHPPATPNNMGLIAGAVGGSLLAALVICGIVYWMHRRTRKAPKRIRLPHIREDDQPSSHQPLFY

SEQ ID NO: 17 - DNA, 60 bp, Artificial Sequence
  gD-rpsL For
cccaggcctaccagcagggggtgacggtggacagcatcgggatgctgcccggcctggtga

SEQ ID NO: 18 - DNA, 88 bp, Artificial Sequence
  gD-rpsL Rev
ccggcgatcttcaagctgtatacggcgacggtgcgctggttctcggggattcagaagaactcgtcaagaaggcgtgatggcgggatcg

SEQ ID NO: 19 - DNA, 106 bp, Artificial Sequence
  gD R222N_F223I_mutant
cccaggcctaccagcagggggtgacggtggacagcatcgggatgctgcccaatatcatccccgagaaccagcgcaccgtcgccgtatacagcttgaagatcgccgg

SEQ ID NO: 20 - DNA, 74 bp, Artificial Sequence
  UL26/27-rpsL_For
gcgtgggggggaggaaatcggcactgaccaagggggtccgttttgtcacgtcagaagaactcgtcaagaaggcg

SEQ ID NO: 21 - DNA, 74 bp, Artificial Sequence
  UL26/27-rpsL_Rev
aacacataaactcccccgggtgtccgcggcctgtttcctctttcctttccggcctggtgatgatggcgggatcg

SEQ ID NO: 22 - DNA, 74 bp, Artificial Sequence
  UL26/27-tkpA_For
gcgtgggggggaggaaatcggcactgaccaagggggtccgttttgtcacggcctcagaagccatagagcccacc

SEQ ID NO: 23 - DNA, 74 bp, Artificial Sequence
  UL26/27-pCMV_Rev
aacacataaactcccccgggtgtccgcggcctgtttcctctttcctttcctatacgcgttgacattgattattg

SEQ ID NO: 24 - protein, 15 aa, Artificial Sequence
  HER2 Linker
GGGGSGGGGSGGGGS

SEQ ID NO: 25 - protein, 27 aa, Artificial Sequence
  EpCAM Linker
ATPSHNSHQVPSAGGPTANSGTSGSEV

SEQ ID NO: 26 - protein, 20 aa, Artificial Sequence
  scFv leader sequence
MSVPTQVLGLLLLWLTGARC

SEQ ID NO: 27 - protein, 351 aa, Artificial Sequence
  Whole sequence _ HER2scFv-HveA adapter
MSVPTQVLGLLLLWLTGARCEVQLVESGGGLVQPGGSLRLSCAASGFNIKDTYIHWVRQAPGKGLEWVARIYPTNGYTRYADSVKGRFTISADTSKNTAYLQMNSLRAEDTAVYYCSRWGGDGFYAMDYWGQGTLVTVSSGGGGSGGGGSGGGGSDIQMTQSPSSLSASVGDRVTITCRASQDVNTAVAWYQQKPGKAPKLLIYSASFLYSGVPSRFSGSRSGTDFTLTISSLQPEDFATYYCQQHYTTPPTFGQGTKVEIKGGGGSEFLPSCKEDEYPVGSECCPKCSPGYRVKEACGELTGTVCEPCPPGTYIAHLNGLSKCLQCQMCDPAMGLRASRNCSRTENAVCG

SEQ ID NO: 28 - DNA, 1053 bp, Artificial Sequence
  Whole sequence _ HER2scFv-HveA adapter
atgagtgtgcccactcaggtcctggggttgctgctgctgtggcttacaggtgccagatgtgaggtgcagctggttgaatctggcggaggactggttcagcctggcggatctctgagactgtcttgtgccgccagcggcttcaacatcaaggacacctacatccactgggtccgacaggcccctggcaaaggacttgaatgggtcgccagaatctaccccaccaacggctacaccagatacgccgactctgtgaagggcagattcaccatcagcgccgacaccagcaagaacaccgcctacctgcagatgaacagcctgagagccgaggacaccgccgtgtactactgttctagatggggaggcgacggcttctacgccatggattattggggccagggcaccctggtcacagtttctagcggaggcggaggttctggcggcggaggaagtggtggcggaggctctgatatccagatgacacagagccccagcagcctgtctgcctctgtgggagacagagtgaccatcacctgtagagccagccaggacgtgaacacagccgtggcttggtatcagcagaagcctggcaaggcccctaagctgctgatctacagcgccagctttctgtacagcggcgtgcccagcagattcagcggctctagaagcggcaccgacttcaccctgaccataagcagtctgcagcccgaggacttcgccacctactactgtcagcagcactacaccacacctccaaccttcggacagggcaccaaggtggaaatcaagggtggtggcggttcagaattcctgccgtcctgcaaggaggacgagtacccagtgggctccgagtgctgccccaagtgcagtccaggttatcgtgtgaaggaggcctgcggggagctgacgggcacagtgtgtgaaccctgccctccaggcacctacattgcccacctcaatggcctaagcaagtgtctgcagtgccaaatgtgtgacccagccatgggcctgcgcgcgagccggaactgctccaggacagagaacgccgtgtgtggc

SEQ ID NO: 29 - protein, 369 aa, Artificial Sequence
  Whole sequence _ EpCAMscFv-HveA adapter
MSVPTQVLGLLLLWLTGARCDIQMTQSPSSLSASVGDRVTITCRSTKSLLHSNGITYLYWYQQKPGKAPKLLIYQMSNLASGVPSRFSSSGSGTDFTLTISSLQPEDFATYYCAQNLEIPRTFGQGTKVELKRATPSHNSHQVPSAGGPTANSGTSGSEVQLVQSGPGLVQPGGSVRISCAASGYTFTNYGMNWVKQAPGKGLEWMGWINTYTGESTYADSFKGRFTFSLDTSASAAYLQINSLRAEDTAVYYCARFAIKGDYWGQGTLLTVSSGGGGSEFLPSCKEDEYPVGSECCPKCSPGYRVKEACGELTGTVCEPCPPGTYIAHLNGLSKCLQCQMCDPAMGLRASRNCSRTENAVCGHHHHHH

SEQ ID NO: 30 - DNA, 1089 bp, Artificial Sequence
  Whole sequence _ EpCAMscFv-HveA adapter
atgagtgtgcccactcaggtcctggggttgctgctgctgtggcttacaggtgccagatgtgatatccagatgacccagtccccgtcctccctgagtgcttctgttggtgaccgtgttaccatcacctgccgttccaccaaatccctcctgcactccaacggtatcacctacctttattggtatcaacagaaaccgggtaaagctccgaaacttctgatctaccagatgtccaacctggcttccggtgttccgtctcgtttctccagttctggttctggtaccgacttcaccctgaccatctcttctctgcagccggaagacttcgctacctactactgcgctcagaacctggaaatcccgcgtaccttcggtcagggtaccaaagttgaacttaagcgcgctaccccgtctcacaactcccaccaggttccatccgcaggcggtccgactgctaactctggaactagtggatccgaagtacagctggttcagtccggcccgggtcttgttcaaccgggtggttccgttcgtatctcttgcgctgcttctggttacacgttcaccaactacggcatgaactgggtcaaacaggctccgggtaaaggcctggaatggatgggctggatcaacacctacaccggtgaatccacctacgctgactccttcaaaggtcgcttcactttctccctcgacacaagtgctagtgctgcatacctccaaatcaactcgctgcgtgcagaggatacagcagtctattactgcgcccgtttcgctatcaaaggtgactactggggtcaaggcacgctgctgaccgtttcctcgggtggtggcggttcagaattcctgccgtcctgcaaggaggacgagtacccagtgggctccgagtgctgccccaagtgcagtccaggttatcgtgtgaaggaggcctgcggggagctgacgggcacagtgtgtgaaccctgccctccaggcacctacattgcccacctcaatggcctaagcaagtgtctgcagtgccaaatgtgtgacccagccatgggcctgcgcgcgagccggaactgctccaggacagagaacgccgtgtgtggc

SEQ ID NO: 31 - DNA, 79 bp, Artificial Sequence
  UL3/4-rpsL-neo_for
taaataacacataaatttggctggttgtttgttgtctttaatggaccgcccgcaaggcctggtgatgatggcgggatcg

SEQ ID NO: 32 - DNA, 78 bp, Artificial Sequence
  UL3/4-rpsL-neo_rev
taggatcccggccggatcgcgctcgtcacccgacactgaaacgccccccccccctcagaagaactcgtcaagaaggcg

SEQ ID NO: 33 - DNA, 79 bp, Artificial Sequence
  UL3/4-HM_pCMV_For
taaataacacataaatttggctggttgtttgttgtctttaatggaccgcccgcaatatacgcgttgacattgattattg

SEQ ID NO: 34 - DNA, 78 bp, Artificial Sequence
  UL3/4_bGH_poly_R
taggatcccggccggatcgcgctcgtcacccgacactgaaacgcccccccccccgcctcagaagccatagagcccacc

SEQ ID NO: 35 - protein, 13 aa, Artificial Sequence
  HER2scFv _ N terminus linker
AAASSGGGSGSGG

SEQ ID NO: 36 - protein, 12 aa, Artificial Sequence
  HER2scFv _ C terminus linker
SGGGSGSGGAAA

SEQ ID NO: 37 - protein, 267 aa, Artificial Sequence
  Whole sequence _ HER2scFv ligand
AAASSGGGSGSGGEVQLVESGGGLVQPGGSLRLSCAASGFNIKDTYIHWVRQAPGKGLEWVARIYPTNGYTRYADSVKGRFTISADTSKNTAYLQMNSLRAEDTAVYYCSRWGGDGFYAMDYWGQGTLVTVSSGGGGSGGGGSGGGGSDIQMTQSPSSLSASVGDRVTITCRASQDVNTAVAWYQQKPGKAPKLLIYSASFLYSGVPSRFSGSRSGTDFTLTISSLQPEDFATYYCQQHYTTPPTFGQGTKVEIKSGGGSGSGGAAA

SEQ ID NO: 38 - DNA, 801 bp, Artificial Sequence
  Whole sequence _ HER2scFv ligand
gcggccgccagtagtggcggtggctctggttccggtggagaggtgcagctggttgaatctggcggaggactggttcagcctggcggatctctgagactgtcttgtgccgccagcggcttcaacatcaaggacacctacatccactgggtccgacaggcccctggcaaaggacttgaatgggtcgccagaatctaccccaccaacggctacaccagatacgccgactctgtgaagggcagattcaccatcagcgccgacaccagcaagaacaccgcctacctgcagatgaacagcctgagagccgaggacaccgccgtgtactactgttctagatggggaggcgacggcttctacgccatggattattggggccagggcaccctggtcacagtttctagcggaggcggaggttctggcggcggaggaagtggtggcggaggctctgatatccagatgacacagagccccagcagcctgtctgcctctgtgggagacagagtgaccatcacctgtagagccagccaggacgtgaacacagccgtggcttggtatcagcagaagcctggcaaggcccctaagctgctgatctacagcgccagctttctgtacagcggcgtgcccagcagattcagcggctctagaagcggcaccgacttcaccctgaccataagcagtctgcagcccgaggacttcgccacctactactgtcagcagcactacaccacacctccaaccttcggacagggcaccaaggtggaaatcaagggtggaggctctggttccggtggatccgcggccgcg

SEQ ID NO: 39 - DNA, 73 bp, Artificial Sequence
  gH29/30-rpsL-neo_For
tcgtgggggttattcttttgggcgttgcgtggggtcaggtccacgactggggcctggtgatgatggcgggatc

SEQ ID NO: 40 - DNA, 74 bp, Artificial Sequence
  gH29/30-rpsL-neo_Rev
ttcgtgtcgcgccagtacatgcggtccatgcccaggccatccaaaaaccatcagaagaactcgtcaagaaggcg

SEQ ID NO: 41 - DNA, 22 bp, Artificial Sequence
  gH29/30-scFv_For
tcgtgggggttattcttttggg

SEQ ID NO: 42 - DNA, 21 bp, Artificial Sequence
  gH29/30-scFv_Rev
ttcgtgtcgcgccagtacatg

SEQ ID NO: 43 - protein, 12 aa, Artificial Sequence
  EpCAMscFv - N terminus linker
AAASSGGGSGSG

SEQ ID NO: 44 - protein, 14 aa, Artificial Sequence
  EpCAMscFv - C terminus linker
SSGGGSGSGGSAAA

SEQ ID NO: 45 - protein, 280 aa, Artificial Sequence
  Whole sequence - EpCAMscFv ligand
AAASSGGGSGSGDIQMTQSPSSLSASVGDRVTITCRSTKSLLHSNGITYLYWYQQKPGKAPKLLIYQMSNLASGVPSRFSSSGSGTDFTLTISSLQPEDFATYYCAQNLEIPRTFGQGTKVELKRATPSHNSHQVPSAGGPTANSGTSGSEVQLVQSGPGLVQPGGSVRISCAASGYTFTNYGMNWVKQAPGKGLEWMGWINTYTGESTYADSFKGRFTFSLDTSASAAYLQINSLRAEDTAVYYCARFAIKGDYWGQGTLLTVSSSSGGGSGSGGSAAA

SEQ ID NO: 46 - DNA, 840 bp, Artificial Sequence
  Whole sequence - EpCAMscFv ligand
gcggccgccagtagtggcggtggctctggttccggtgatatccagatgacccagtccccgtcctccctgagtgcttctgttggtgaccgtgttaccatcacctgccgttccaccaaatccctcctgcactccaacggtatcacctacctttattggtatcaacagaaaccgggtaaagctccgaaacttctgatctaccagatgtccaacctggcttccggtgttccgtctcgtttctccagttctggttctggtaccgacttcaccctgaccatctcttctctgcagccggaagacttcgctacctactactgcgctcagaacctggaaatcccgcgtaccttcggtcagggtaccaaagttgaacttaagcgcgctaccccgtctcacaactcccaccaggttccatccgcaggcggtccgactgctaactctggaactagtggatccgaagtacagctggttcagtccggcccgggtcttgttcaaccgggtggttccgttcgtatctcttgcgctgcttctggttacacgttcaccaactacggcatgaactgggtcaaacaggctccgggtaaaggcctggaatggatgggctggatcaacacctacaccggtgaatccacctacgctgactccttcaaaggtcgcttcactttctccctcgacacaagtgctagtgctgcatacctccaaatcaactcgctgcgtgcagaggatacagcagtctattactgcgcccgtttcgctatcaaaggtgactactggggtcaaggcacgctgctgaccgtttcctcgtcttccggtggaggctctggttccggtggatccgcggccgcg